European Patent Specification EP 3 568 411 B1, published March 6, 2024. Title: METHODS AND COMPOSITIONS FOR TREATING HPA HYPERACTIVITY. Applicant: SANNA, PIETRO P. LLOYD, LINDA S. The sequence listing filed with the application follows.

SEQUENCE LISTING (66 sequences)

SEQ ID NO: 1 - protein, 322 aa, Homo sapiens
MSPNFKLQCHFILIFLTALRGESRYLELREAADYDPFLLFSANLKRELAGEQPYRRALRCLDMLSLQGQFTFTADRPQLHCAAFFISEPEEFITIHYDQVSIDCQGGDFLKVFDGWILKGEKFPSSQDHPLPSAERYIDFCESGLSRRSIRSSQNVAMIFFRVHEPGNGFTLTIKTDPNLFPCNVISQTPNGKFTLVVPHQHRNCSFSIIYPVVIKISDLTLGHVNGLQLKKSSAGCEGIGDFVELLGGTGLDPSKMTPLADLCYPFHGPAQMKVGCDNTVVRMVSSGKHVNRVTFEYRQLEPYELENPNGNSIGEFCLSGL

SEQ ID NO: 2 - protein, 322 aa, Mus musculus
MSPNFKLQCHFILILLTALRGESRYLEVQEAAVYDPLLLFSANLKRDLAEEQPYRRALRCLDMLSLPGQFTFTADRPQLHCAAFFIGEPEEFITIHYDLVSIDCQGGDFLKVFDGWILKGEKFPSSQDHPLPTMKRYTDFCESGLTRRSIRSSQNVAMVFFRVHEPGNGFTITIKTDPNLFPCNVISQTPSGRFTLVVPYQHQNCSFSIIYPVAIKISDLTLGHLHGLQLKKPAAGCGGTGDFVELLGGTGLDPSKMMPLADLCYPFLGPAQMKISCDNAVVRMVSSGKHINRVTFEYRQLEPFELETSTGNSIPEYCLSSL

SEQ ID NO: 3 - protein, 355 aa, Gallus gallus
MPRRLLPAGSEQQVLSAHGGAATMPSAFQLQCHLVLILLAASKGDTRYLEVRDAGEDEPFLLLSEDLKRELSAGHIYRRSLRRAEPSPVSAGCIDMLSIEGQFTFTADQPQLHCATFFIGEPEELLTIEYDFVNIDCQGGDFLKVFDGWILKGEKFPSSLDHPLPTSQRYTDFCESGAVQRSIRSSQNVAMIFFRIHQPGNGFTITVKKSANLFPCNVISQTPSGRFTMVIPHQHRNCSFSIIYPVVIKISDLILGHLNGLFLKNPSVGCAGVGDFVELLGGTGLDPSKMFPLADLCHSFHGSAQMKIGCDNTVLRMVSSGKHINRVTFEYYQLDLQEIENRKENSIEEFCFPGI

SEQ ID NO: 4 - protein, 321 aa, Xenopus laevis
MTPASRPDWCLILLFLAVLRGESRYIQMREAAEDALFLLNSDFKRELSEGQIYRRSLRCIDMLSIEGQFTFQADRPQLHCALFLIGEPEEFIIIEYNFVNIDCIGGDILKVFDGWIIKGEKFPSSLDHPLSTMERYTDICEDGDVGSITRSSQNVAMIFFRVQQPGHGFTLTIRKIPNLFPCNVISQSMNGRFTMITPHQHRNCSFSIIYPVVIKIFDLTLGHFNELQLKKPPPKGCGDAGDFVELLGGAGLDPSKMFPLADLCHSFHGSAQMKIGCDNTVVRMVSSGNFINRVTFEYNQLDRQLEKKQGNSVEEACFPSD

SEQ ID NO: 5 - protein, 321 aa, Cyprinus carpio
MSGTSRAQLCFLLLSVTALRGHARFLDIQDNEISPEGLLSLLSSELKRELPEEFVYRRALRCLDMVAIEGQFTFTAERPQLNCAVFFIGEPSDIISIEYDSVNIDCRGGDFIKVFDGWVMKGEKFPSTQDHPLPLYKRYSDYCETGVTRPIVRSSQNVAMLFFRLHQSGSSFTVTFRKLINPFPCNVVSQTPEGSFTMIIPQQHRNCSFSIIYPVEIQIGELSLGQHNDLKRSILGCAGSGDFVELLGGNGMDTSKMYPMADLCYSFNGPAQMKVGCDNTVIRMVSSGKFVNRVSFQYRLLGHQELQQMKGNSVEDVCLRA

SEQ ID NO: 6 - protein, 332 aa, Apis mellifera
MFLNGSLYCFARLFFIIGFFNAISGAIKGNDYQRYHQQISGDRFSKDFYRQDTKNNLLNAYVRFKLVTDCIFVTSEPGYFLYTSKNDNEEVCGIYFLAEPDQKIEINFITFDIPCEHRGLVSIIDGWELNGEVFPSKMDHQLPLKQRSSEFCGKNIGMKRIFTSSQNIAVIEYRIPKSGKGFSLFARFLKNPRPCNVLATSLTEPYTLRNYGRRINCTYVALYPSSVQVIALGVGVSNFLSSTRTAETGTIRKCDESSPHDQVIIGGSNGLDTSKVHIIDSICGIDSKPDYRELTEYSVTSVRLISSGFFDNFVTVQIQPLKNELFNANIGI

SEQ ID NO: 7 - protein, 33 aa, Artificial Sequence
  source: /note="Description of Artificial Sequence: Synthetic polypeptide"
DLTFHLLREMLEMAKAEQEAEQAALNRLLLEEA

SEQ ID NO: 8 - protein, 30 aa, Artificial Sequence
  source: /note="Description of Artificial Sequence: Synthetic polypeptide"
  MOD_RES (1)..(1): D-amino acid
  MOD_RES (10)..(10): Nle
  MISC_FEATURE (19)..(22): /note="Cyclic"
  VARIANT (27)..(27): /replace="Nle"
  MISC_FEATURE (1)..(30): /note="Variant residues given in the sequence have no preference with respect to those in the annotations for variant positions"
FLLLLGLNPXSASLQDQHEESLSLASKISG

SEQ ID NO: 9 - protein, 6 aa, Artificial Sequence
  source: /note="Description of Artificial Sequence: Synthetic peptide"
GSEGEG

SEQ ID NO: 10 - protein, 20 aa, Artificial Sequence
  source: /note="Description of Artificial Sequence: Synthetic peptide"
AESPGPGTSPSGESSTAPGT

SEQ ID NO: 11 - protein, 5 aa, Artificial Sequence
  source: /note="Description of Artificial Sequence: Synthetic peptide"
GGGGS

SEQ ID NO: 12 - protein, 210 aa, Homo sapiens
YLELREAADYDPFLLFSANLKRELAGEQPYRRALRCLDMLSLQGQFTFTADRPQLHCAAFFISEPEEFITIHYDQVSIDCQGGDFLKVFDGWILKGEKFPSSQDHPLPSAERYIDFCESGLSRRSIRSSQNVAMIFFRVHEPGNGFTLTIKTDPNLFPCNVISQTPNGKFTLVVPHQHRNCSFSIIYPVVIKISDLTLGHVNGLQLKKSS

SEQ ID NO: 13 - protein, 298 aa, Homo sapiens
YLELREAADYDPFLLFSANLKRELAGEQPYRRALRCLDMLSLQGQFTFTADRPQLHCAAFFISEPEEFITIHYDQVSIDCQGGDFLKVFDGWILKGEKFPSSQDHPLPSAERYIDFCESGLSRRSIRSSQNVAMIFFRVHEPGNGFTLTIKTDPNLFPCNVISQTPNGKFTLVVPHQHRNCSFSIIYPVVIKISDLTLGHVNGLQLKKSSAGCEGIGDFVELLGGTGLDPSKMTPLADLCYPFHGPAQMKVGCDNTVVRMVSSGKHVNRVTFEYRQLEPYELENPNGNSIGEFCLSGL

SEQ ID NO: 14 - protein, 210 aa, Rattus norvegicus
YLEVQEAAVYDPFLLFSANLKRNLAEEQPYRRALRCLDMLSLPGQFTFTADQPQLHCAAFFIGEPEEFITIHFDLVSIDCQGGDFLKVFDGWILKGEKFPSSQDHPLPTRERYTDFCESGLTRRSVTSSQNVAMVFFRVHEPGNGFTITIKTDPNLFPCNIISQTPSGRFALVVPYQHQNCSFSIIYPVTIKISDLALGHLHGLQLKKPA

SEQ ID NO: 15 - protein, 298 aa, Rattus norvegicus
YLEVQEAAVYDPFLLFSANLKRNLAEEQPYRRALRCLDMLSLPGQFTFTADQPQLHCAAFFIGEPEEFITIHFDLVSIDCQGGDFLKVFDGWILKGEKFPSSQDHPLPTRERYTDFCESGLTRRSVTSSQNVAMVFFRVHEPGNGFTITIKTDPNLFPCNIISQTPSGRFALVVPYQHQNCSFSIIYPVTIKISDLALGHLHGLQLKKPAAGCGGTGDFVELLGGTGLDTSKMMLLVDLCYPFHGPAQMKISCDNAVVRMVSSGKHMNRVTFEYRQLEPLELETSTRNSIPEYCLSSL

SEQ ID NO: 16 - protein, 546 aa, Mus musculus
MSPNFKLQCHFILIFLTALRGESRYLELREAADYDPFLLFSANLKRELAGEQPYRRALRCLDMLSLQGQFTFTADRPQLHCAAFFISEPEEFITIHYDQVSIDCQGGDFLKVFDGWILKGEKFPSSQDHPLPSAERYIDFCESGLSRRSIRSSQNVAMIFFRVHEPGNGFTLTIKTDPNLFPCNVISQTPNGKFTLVVPHQHRNCSFSIIYPVVIKISDLTLGHVNGLQLKKSSAGCEGIGDFVELLGGTGLDPSKMTPLADLCYPFHGPAQMKVGCDNTVVRMVSSGKHVNRVTFEYRQLEPYELENPNGNSIGEFCLSGLTGGCKPCICTVPEVSSVFIFPPKPKDVLTITLTPKVTCVVVDISKDDPEVQFSWFVDDVEVHTAQTQPREEQFNSTFRSVSELPIMHQDWLNGKEFKCRVNSAAFPAPIEKTISKTKGRPKAPQVYTIPPPKEQMAKDKVSLTCMITDFFPEDITVEWQWNGQPAENYKNTQPIMDTDGSYFVYSKLNVQKSNWEAGNTFTCSVLHEGLHNHHTEKSLSHSPGK

SEQ ID NO: 17 - protein, 458 aa, Mus musculus
MSPNFKLQCHFILIFLTALRGESRYLELREAADYDPFLLFSANLKRELAGEQPYRRALRCLDMLSLQGQFTFTADRPQLHCAAFFISEPEEFITIHYDQVSIDCQGGDFLKVFDGWILKGEKFPSSQDHPLPSAERYIDFCESGLSRRSIRSSQNVAMIFFRVHEPGNGFTLTIKTDPNLFPCNVISQTPNGKFTLVVPHQHRNCSFSIIYPVVIKISDLTLGHVNGLQLKKSSTGGCKPCICTVPEVSSVFIFPPKPKDVLTITLTPKVTCVVVDISKDDPEVQFSWFVDDVEVHTAQTQPREEQFNSTFRSVSELPIMHQDWLNGKEFKCRVNSAAFPAPIEKTISKTKGRPKAPQVYTIPPPKEQMAKDKVSLTCMITDFFPEDITVEWQWNGQPAENYKNTQPIMDTDGSYFVYSKLNVQKSNWEAGNTFTCSVLHEGLHNHHTEKSLSHSPGK

SEQ ID NO: 18 - protein, 332 aa, Artificial Sequence
  source: /note="Description of Artificial Sequence: Synthetic polypeptide"
MSPNFKLQCHFILIFLTALRGESRYLELREAADYDPFLLFSANLKRELAGEQPYRRALRCLDMLSLQGQFTFTADRPQLHCAAFFISEPEEFITIHYDQVSIDCQGGDFLKVFDGWILKGEKFPSSQDHPLPSAERYIDFCESGLSRRSIRSSQNVAMIFFRVHEPGNGFTLTIKTDPNLFPCNVISQTPNGKFTLVVPHQHRNCSFSIIYPVVIKISDLTLGHVNGLQLKKSSAGCEGIGDFVELLGGTGLDPSKMTPLADLCYPFHGPAQMKVGCDNTVVRMVSSGKHVNRVTFEYRQLEPYELENPNGNSIGEFCLSGLGTDYKDDDDK

SEQ ID NO: 19 - protein, 332 aa, Artificial Sequence
  source: /note="Description of Artificial Sequence: Synthetic polypeptide"
MSPNFKLQCHFILIFLTALRGESRYLELREAADYDPFLLFSANLKRELAGEQPYRRALRCLDMLSLQGQFTFTADRPQLHCAAFFISEPEEFITIHYDQVSIDCQGGDFLKVFDGWILKGEKFPSSQDHPLPSAERYIDFCESGLSRRSIRSSQNVAMIFFRVHEPGNGFTLTIKTDPNLFPCNVISQTPNGKFTLVVPHQHRNCSFSIIYPVVIKISDLTLGHVNGLQLKKSSAGCEGIGDFVELLGGTGLDPSKMTPLADLCYPFHGPAQMKVGCDNTVVRMVSSGKHVNRVTFEYRQLEPYELENPNGNSIGEFCLSGLGTWSHPQFEK

SEQ ID NO: 20 - protein, 342 aa, Artificial Sequence
  source: /note="Description of Artificial Sequence: Synthetic polypeptide"
MSPNFKLQCHFILIFLTALRGESRYLELREAADYDPFLLFSANLKRELAGEQPYRRALRCLDMLSLQGQFTFTADRPQLHCAAFFISEPEEFITIHYDQVSIDCQGGDFLKVFDGWILKGEKFPSSQDHPLPSAERYIDFCESGLSRRSIRSSQNVAMIFFRVHEPGNGFTLTIKTDPNLFPCNVISQTPNGKFTLVVPHQHRNCSFSIIYPVVIKISDLTLGHVNGLQLKKSSAGCEGIGDFVELLGGTGLDPSKMTPLADLCYPFHGPAQMKVGCDNTVVRMVSSGKHVNRVTFEYRQLEPYELENPNGNSIGEFCLSGLGTDYKDDDDKEFWSHPQFEK

SEQ ID NO: 21 - protein, 556 aa, Artificial Sequence
  source: /note="Description of Artificial Sequence: Synthetic polypeptide"
MSPNFKLQCHFILIFLTALRGESRYLELREAADYDPFLLFSANLKRELAGEQPYRRALRCLDMLSLQGQFTFTADRPQLHCAAFFISEPEEFITIHYDQVSIDCQGGDFLKVFDGWILKGEKFPSSQDHPLPSAERYIDFCESGLSRRSIRSSQNVAMIFFRVHEPGNGFTLTIKTDPNLFPCNVISQTPNGKFTLVVPHQHRNCSFSIIYPVVIKISDLTLGHVNGLQLKKSSAGCEGIGDFVELLGGTGLDPSKMTPLADLCYPFHGPAQMKVGCDNTVVRMVSSGKHVNRVTFEYRQLEPYELENPNGNSIGEFCLSGLGSGGGGSGGGGSGCKPCICTVPEVSSVFIFPPKPKDVLTITLTPKVTCVVVDISKDDPEVQFSWFVDDVEVHTAQTQPREEQFNSTFRSVSELPIMHQDWLNGKEFKCRVNSAAFPAPIEKTISKTKGRPKAPQVYTIPPPKEQMAKDKVSLTCMITDFFPEDITVEWQWNGQPAENYKNTQPIMDTDGSYFVYSKLNVQKSNWEAGNTFTCSVLHEGLHNHHTEKSLSHSPGK

SEQ ID NO: 22 - protein, 575 aa, Artificial Sequence
  source: /note="Description of Artificial Sequence: Synthetic polypeptide"
MSPNFKLQCHFILIFLTALRGESRYLELREAADYDPFLLFSANLKRELAGEQPYRRALRCLDMLSLQGQFTFTADRPQLHCAAFFISEPEEFITIHYDQVSIDCQGGDFLKVFDGWILKGEKFPSSQDHPLPSAERYIDFCESGLSRRSIRSSQNVAMIFFRVHEPGNGFTLTIKTDPNLFPCNVISQTPNGKFTLVVPHQHRNCSFSIIYPVVIKISDLTLGHVNGLQLKKSSAGCEGIGDFVELLGGTGLDPSKMTPLADLCYPFHGPAQMKVGCDNTVVRMVSSGKHVNRVTFEYRQLEPYELENPNGNSIGEFCLSGLGSGGGGSGGGGSGGGGSGGGSGGGGSGGGGSGCKPCICTVPEVSSVFIFPPKPKDVLTITLTPKVTCVVVDISKDDPEVQFSWFVDDVEVHTAQTQPREEQFNSTFRSVSELPIMHQDWLNGKEFKCRVNSAAFPAPIEKTISKTKGRPKAPQVYTIPPPKEQMAKDKVSLTCMITDFFPEDITVEWQWNGQPAENYKNTQPIMDTDGSYFVYSKLNVQKSNWEAGNTFTCSVLHEGLHNHHTEKSLSHSPGK

SEQ ID NO: 23 - protein, 575 aa, Artificial Sequence
  source: /note="Description of Artificial Sequence: Synthetic polypeptide"
MYRMQLLSCIALSLALVTNSYLELREAADYDPFLLFSANLKRELAGEQPYRRALRCLDMLSLQGQFTFTADRPQLHCAAFFISEPEEFITIHYDQVSIDCQGGDFLKVFDGWILKGEKFPSSQDHPLPSAERYIDFCESGLSRRSIRSSQNVAMIFFRVHEPGNGFTLTIKTDPNLFPCNVISQTPNGKFTLVVPHQHRNCSFSIIYPVVIKISDLTLGHVNGLQLKKSSAGCEGIGDFVELLGGTGLDPSKMTPLADLCYPFHGPAQMKVGCDNTVVRMVSSGKHVNRVTFEYRQLEPYELENPNGNSIGEFCLSGLGSGGGGSGGGGSGGGGSGGGGSGGGGSGGGGSRSVECPPCPAPPVAGPSVFLFPPKPKDTLMISRTPEVTCVVVDVSHEDPEVQFNWYVDGVEVHNAKTKPREEQFNSTFRVVSVLTVVHQDWLNGKEYKCKVSNKGLPAPIEKTISKTKGQPREPQVYTLPPSREEMTKNQVSLTCLVKGFYPSDIAVEWESNGQPENNYKTTPPMLDSDGSFFLYSKLTVDKSRWQQGNVFSCSVMHEALHNHYTQKSLSLSPGK

SEQ ID NO: 24 - protein, 487 aa, Artificial Sequence
  source: /note="Description of Artificial Sequence: Synthetic polypeptide"
MYRMQLLSCIALSLALVTNSYLELREAADYDPFLLFSANLKRELAGEQPYRRALRCLDMLSLQGQFTFTADRPQLHCAAFFISEPEEFITIHYDQVSIDCQGGDFLKVFDGWILKGEKFPSSQDHPLPSAERYIDFCESGLSRRSIRSSQNVAMIFFRVHEPGNGFTLTIKTDPNLFPCNVISQTPNGKFTLVVPHQHRNCSFSIIYPVVIKISDLTLGHVNGLQLKKSSGSGGGGSGGGGSGGGGSGGGGSGGGGSGGGGSRSVECPPCPAPPVAGPSVFLFPPKPKDTLMISRTPEVTCVVVDVSHEDPEVQFNWYVDGVEVHNAKTKPREEQFNSTFRVVSVLTVVHQDWLNGKEYKCKVSNKGLPAPIEKTISKTKGQPREPQVYTLPPSREEMTKNQVSLTCLVKGFYPSDIAVEWESNGQPENNYKTTPPMLDSDGSFFLYSKLTVDKSRWQQGNVFSCSVMHEALHNHYTQKSLSLSPGK

SEQ ID NO: 25 - protein, 5 aa, Artificial Sequence
  source: /note="Description of Artificial Sequence: Synthetic peptide"
KSSAG

SEQ ID NO: 26 - protein, 7 aa, Artificial Sequence
  source: /note="Description of Artificial Sequence: Synthetic peptide"
KKSSAGC

SEQ ID NO: 27 - protein, 6 aa, Artificial Sequence
  source: /note="Description of Artificial Sequence: Synthetic peptide"
  MOD_RES (1)..(2): Any amino acid
  MOD_RES (4)..(5): Any amino acid
XXNXXG

SEQ ID NO: 28 - protein, 4 aa, Artificial Sequence
  source: /note="Description of Artificial Sequence: Synthetic peptide"
GGGG

SEQ ID NO: 29 - protein, 5 aa, Artificial Sequence
  source: /note="Description of Artificial Sequence: Synthetic peptide"
GGGGG

SEQ ID NO: 30 - protein, 7 aa, Artificial Sequence
  source: /note="Description of Artificial Sequence: Synthetic peptide"
GGGGGGG

SEQ ID NO: 31 - protein, 6 aa, Artificial Sequence
  source: /note="Description of Artificial Sequence: Synthetic peptide"
GGGGGK

SEQ ID NO: 32 - protein, 7 aa, Artificial Sequence
  source: /note="Description of Artificial Sequence: Synthetic peptide"
GGGGGKR

SEQ ID NO: 33 - protein, 8 aa, Artificial Sequence
  source: /note="Description of Artificial Sequence: Synthetic peptide"
GGGKGGGG

SEQ ID NO: 34 - protein, 8 aa, Artificial Sequence
  source: /note="Description of Artificial Sequence: Synthetic peptide"
GGGNGSGG

SEQ ID NO: 35 - protein, 8 aa, Artificial Sequence
  source: /note="Description of Artificial Sequence: Synthetic peptide"
GGGCGGGG

SEQ ID NO: 36 - protein, 5 aa, Artificial Sequence
  source: /note="Description of Artificial Sequence: Synthetic peptide"
GPNGG

SEQ ID NO: 37 - protein, 8 aa, Artificial Sequence
  source: /note="Description of Artificial Sequence: Synthetic peptide"
GGGKGGGG

SEQ ID NO: 38 - protein, 10 aa, Artificial Sequence
  source: /note="Description of Artificial Sequence: Synthetic peptide"
GGGGSGGGGS

SEQ ID NO: 39 - protein, 25 aa, Artificial Sequence
  source: /note="Description of Artificial Sequence: Synthetic peptide"
GGGGSGGGGSGGGGSGGGGSGGGGS

SEQ ID NO: 40 - protein, 6 aa, Artificial Sequence
  source: /note="Description of Artificial Sequence: Synthetic peptide"
GGEGGG

SEQ ID NO: 41 - protein, 8 aa, Artificial Sequence
  source: /note="Description of Artificial Sequence: Synthetic peptide"
GGEEEGGG

SEQ ID NO: 42 - protein, 5 aa, Artificial Sequence
  source: /note="Description of Artificial Sequence: Synthetic peptide"
GEEEG

SEQ ID NO: 43 - protein, 4 aa, Artificial Sequence
  source: /note="Description of Artificial Sequence: Synthetic peptide"
GEEE

SEQ ID NO: 44 - protein, 6 aa, Artificial Sequence
  source: /note="Description of Artificial Sequence: Synthetic peptide"
GGDGGG

SEQ ID NO: 45 - protein, 7 aa, Artificial Sequence
  source: /note="Description of Artificial Sequence: Synthetic peptide"
GGDDDGG

SEQ ID NO: 46 - protein, 5 aa, Artificial Sequence
  source: /note="Description of Artificial Sequence: Synthetic peptide"
GDDDG

SEQ ID NO: 47 - protein, 4 aa, Artificial Sequence
  source: /note="Description of Artificial Sequence: Synthetic peptide"
GDDD

SEQ ID NO: 48 - protein, 21 aa, Artificial Sequence
  source: /note="Description of Artificial Sequence: Synthetic peptide"
GGGGSDDSDEGSDGEDGGGGS

SEQ ID NO: 49 - protein, 5 aa, Artificial Sequence
  source: /note="Description of Artificial Sequence: Synthetic peptide"
WEWEW

SEQ ID NO: 50 - protein, 5 aa, Artificial Sequence
  source: /note="Description of Artificial Sequence: Synthetic peptide"
FEFEF

SEQ ID NO: 51 - protein, 6 aa, Artificial Sequence
  source: /note="Description of Artificial Sequence: Synthetic peptide"
EEEWWW

SEQ ID NO: 52 - protein, 6 aa, Artificial Sequence
  source: /note="Description of Artificial Sequence: Synthetic peptide"
EEEFFF

SEQ ID NO: 53 - protein, 7 aa, Artificial Sequence
  source: /note="Description of Artificial Sequence: Synthetic peptide"
WWEEEWW

SEQ ID NO: 54 - protein, 7 aa, Artificial Sequence
  source: /note="Description of Artificial Sequence: Synthetic peptide"
FFEEEFF

SEQ ID NO: 55 - protein, 6 aa, Artificial Sequence
  source: /note="Description of Artificial Sequence: Synthetic peptide"
  MOD_RES (1)..(2): Any amino acid
  MOD_RES (4)..(5): Any amino acid
XXYXXG

SEQ ID NO: 56 - protein, 6 aa, Artificial Sequence
  source: /note="Description of Artificial Sequence: Synthetic peptide"
  MOD_RES (1)..(2): Any amino acid
  MOD_RES (4)..(5): Any amino acid
XXSXXG

SEQ ID NO: 57 - protein, 6 aa, Artificial Sequence
  source: /note="Description of Artificial Sequence: Synthetic peptide"
  MOD_RES (1)..(2): Any amino acid
  MOD_RES (4)..(5): Any amino acid
XXTXXG

SEQ ID NO: 58 - protein, 22 aa, Artificial Sequence
  source: /note="Description of Artificial Sequence: Synthetic peptide"
GSGSATGGSGSTASSGSGSATH

SEQ ID NO: 59 - protein, 22 aa, Artificial Sequence
  source: /note="Description of Artificial Sequence: Synthetic peptide"
HGSGSATGGSGSTASSGSGSAT

SEQ ID NO: 60 - protein, 19 aa, Artificial Sequence
  source: /note="Description of Artificial Sequence: Synthetic peptide"
AEAAAKEAAAKEAAAKAGG

SEQ ID NO: 61 - protein, 444 aa, Artificial Sequence
  source: /note="Description of Artificial Sequence: Synthetic polypeptide"
  MOD_RES (13)..(13): D-amino acid
MGGHPQLRLVKAHLLLGLNPVSASLQDQHCESLSLASNISGLQCNASVDLIGTCWPRSPAGQLVVRPCPAFFYGVRYNTTNNGYRECLANGSWAARVNYSECQEILNEEKKSKVHYHVAVIINYLGHCISLVALLVAFVLFLRLRPGCTHWGDQADGALEVGAPWSGAPFQVRRSIRCLRNIIHWNLISAFILRNATWFVVQLTMSPEVHQSNVGWCRLVTAAYNYFHVTNFFWMFGEGCYLHTAIVLTYSTDRLRKWMFICIGWGVPFPIIVAWAIGKLYYDNEKCWFGKRPGVYTDYIYQGPMILVLLINFIFLFNIVRILMTKLRASTTSETIQYRKAVKATLVLLPLLGITYMLFFVNPGEDEVSRVVFIYFNSFLESFQGFFVSVFYCFLNSEVRSAIRKRWHRWQDKHSIRARVARAMSIPTSPTRVSFHSIKQSTAV

SEQ ID NO: 62 - protein, 31 aa, Artificial Sequence
  source: /note="Description of Artificial Sequence: Synthetic polypeptide"
  MOD_RES (1)..(1): D-amino acid
FALLLLGLNPVSASLQDQHCESLSLASNISG

SEQ ID NO: 63 - protein, 298 aa, Artificial Sequence
  source: /note="Description of Artificial Sequence: Synthetic polypeptide"
YLELREAADYDPFLLFSANLKRELAGEQPYRRALRCLDMLSLQGQFTFTADRPQLHCAAFFISEPEEFITIHYDQVSIDCQGGDFLKVFDGWILKGEKFPSSQDHPLPSAERYIDFCESGLSRRSIRSSQNVAMIFFRVHEPGNGFTLTIKTDPNLFPCNVISQTPNGKFTLVVPHQHRNCSFSIIYPVVIKISDLTLGHVNGLQLKKNCSGCEGIGDFVELLGGTGLDPSKMTPLADLCYPFHGPAQMKVGCDNTVVRMVSSGKHVNRVTFEYRQLEPYELENPNGNSIGEFCLSGL

SEQ ID NO: 64 - protein, 30 aa, Homo sapiens
FQSSSSKAPPPSLPSPSRLPGPSDTPILPQ

SEQ ID NO: 65 - protein, 15 aa, Artificial Sequence
  source: /note="Description of Artificial Sequence: Synthetic peptide"
GGGGSGGGGSGGGGS

SEQ ID NO: 66 - protein, 5 aa, Artificial Sequence
  source: /note="Description of Artificial Sequence: Synthetic peptide"
  MOD_RES (4)..(4): Any amino acid except Pro
VPGXG